European Patent Specification EP 4 121 166 B1, published January 31, 2024. Title: Therapeutic treatment of chromatinopathies. Applicant: UNIVERSITA' DEGLI STUDI DI TRENTO. The sequence listing filed with the application follows.

SEQUENCE LISTING (37 sequences)

SEQ ID NO: 1 - DNA, 33 bp, unknown
  sgRNA-F1
aaactcgagtgtacaaaaaagcaggctttaaag

SEQ ID NO: 2 - DNA, 43 bp, unknown
  sgRNA-F2
gtggctgcagctgcagagagcgttttagagctagaaatagcaa

SEQ ID NO: 3 - DNA, 38 bp, unknown
  sgRNA-R1
gctctctgcagctgcagccacggtgtttcgtcctttcc

SEQ ID NO: 4 - DNA, 43 bp, unknown; identical to SEQ ID NO: 2
  sgRNA-F2

SEQ ID NO: 5 - DNA, 32 bp, unknown
  MLL4 PrLD_fwd_BglII
gccagatctggtgatgctgagaagctcaagct

SEQ ID NO: 6 - DNA, 31 bp, unknown
  MLL4 PrLD_rev_SalI_STOP
gccgtcgactttactgtggtccagggaagcc

SEQ ID NO: 7 - DNA, 29 bp, unknown
  MLL4-PrLD ΔQ_revi_
taaagagcccatgggctgagcgctcagtt

SEQ ID NO: 8 - DNA, 50 bp, unknown
  MLL4-PrLD ΔQ_fwdi
gctcagcccatgggctctttttttaaaccagagtcgaactttactgtctc

SEQ ID NO: 9 - DNA, 20 bp, unknown
  GAPDH fwd
aggtgaaggtcggagtcaac

SEQ ID NO: 10 - DNA, 23 bp, unknown
  GAPDH rev
ccatgtagttgaggtcaatgaag

SEQ ID NO: 11 - DNA, 19 bp, unknown
  RING1B fwd
gccaggatcaacaagcaca

SEQ ID NO: 12 - DNA, 19 bp, unknown
  RING1B rev
ttgtttcttgcctcgctgc

SEQ ID NO: 13 - DNA, 20 bp, unknown
  KDM6A fwd
cctctttgggttcgtgagat

SEQ ID NO: 14 - DNA, 22 bp, unknown
  KDM6A rev
gactccacttttccttcagctt

SEQ ID NO: 15 - DNA, 19 bp, unknown
  BMI fwd
tcattgtcttttccgcccg

SEQ ID NO: 16 - DNA, 20 bp, unknown
  BMI rev
tcaggtggggatttagctca

SEQ ID NO: 17 - DNA, 20 bp, unknown
  KMT2D fwd
tgaaagggcactgagggata

SEQ ID NO: 18 - DNA, 18 bp, unknown
  KMT2D rev
tgagggggtgtaggcaag

SEQ ID NO: 19 - DNA, 20 bp, unknown
  LMNA fwd
acccatctcctctggctctt

SEQ ID NO: 20 - DNA, 20 bp, unknown
  LMNA rev
gtgaccagattgtccccgaa

SEQ ID NO: 21 - DNA, 20 bp, unknown
  TOP2B fwd
aggaaagcatctggctctga

SEQ ID NO: 22 - DNA, 20 bp, unknown
  TOP2B rev
tctgaggggaagatgtccac

SEQ ID NO: 23 - DNA, 20 bp, unknown
  SMC4 fwd
tcggttctaagcccagagga

SEQ ID NO: 24 - DNA, 20 bp, unknown
  SMC4 rev
tatactctgcgatggcaccg

SEQ ID NO: 25 - DNA, 20 bp, unknown
  RAD21 fwd
tcccccagaagaacctccaa

SEQ ID NO: 26 - DNA, 20 bp, unknown
  RAD21 rev
acgctgaagaccatgaagca

SEQ ID NO: 27 - DNA, 20 bp, unknown
  TOP2A fwd
tgtcaaaccagttcctgcaa

SEQ ID NO: 28 - DNA, 20 bp, unknown
  TOP2A rev
ctgtgacgaaaccatgttgg

SEQ ID NO: 29 - DNA, 18 bp, unknown
  COL II fwd
caggatgtccaggaggct

SEQ ID NO: 30 - DNA, 22 bp, unknown
  COL II rev
gcttccacacatccttatcatt

SEQ ID NO: 31 - DNA, 21 bp, unknown
  AGC fwd
ggagtccaactcttcaaggtg

SEQ ID NO: 32 - DNA, 25 bp, unknown
  AGC rev
atggtctgaagtttctacagtgaca

SEQ ID NO: 33 - DNA, 20 bp, unknown
  COL10A1 fwd
cccaacaccaagacacagtt

SEQ ID NO: 34 - DNA, 20 bp, unknown
  COL10A1 rev
gtggaccaggagtaccttgc

SEQ ID NO: 35 - DNA, 20 bp, unknown
  MMP13 fwd
gcagctgttcactttgagga

SEQ ID NO: 36 - DNA, 22 bp, unknown
  MMP13 rev
catcatatctccagacctggtt

SEQ ID NO: 37 - DNA, 25 bp, unknown
  MO-Kmt2d
ccctgctgctgctttgatctttttg